European Patent Specification EP 3 708 680 B1, published July 26, 2023. Title: COMPOSITIONS AND METHODS FOR XI CHROMOSOME REACTIVATION. Applicant: University of Massachusetts. Application Not yet assigned. The sequence listing filed with the application follows.

SEQUENCE LISTING (119 sequences)

SEQ ID NO: 1 - DNA, 19 bp, Artificial Sequence
  Synthetic Polynucleotide
ttgccgacaggatgcagaa

SEQ ID NO: 2 - DNA, 20 bp, Mus musculus
ggccagcagtgtttttcttc

SEQ ID NO: 3 - DNA, 20 bp, Homo sapiens
tcaggaagtggctctggtct

SEQ ID NO: 4 - DNA, 20 bp, Mus musculus
taggatactgcttgttactt

SEQ ID NO: 5 - DNA, 20 bp, Homo sapiens
tggaatatgcaccacttgga

SEQ ID NO: 6 - DNA, 22 bp, Artificial Sequence
  Synthetic Polynucleotide
aaatcagggggttgaaaaatct

SEQ ID NO: 7 - DNA, 26 bp, Artificial Sequence
  Synthetic Polynucleotide
gccaagtgaaaaccaggacaaaagac

SEQ ID NO: 8 - DNA, 25 bp, Mus musculus
ggaaggctacctggctaaagtcaag

SEQ ID NO: 9 - DNA, 20 bp, Homo sapiens
gtgggggactgtgtctctgt

SEQ ID NO: 10 - DNA, 20 bp, Artificial Sequence
  Synthetic Polynucleotide
cctggtggtgttttgttgtg

SEQ ID NO: 11 - DNA, 27 bp, Artificial Sequence
  Synthetic Polynucleotide
ctaattggtacttactacgataacttt

SEQ ID NO: 12 - DNA, 20 bp, Mus musculus
gctgagccattttcttctcg

SEQ ID NO: 13 - DNA, 20 bp, Homo sapiens
caagggttgtggagagtggt

SEQ ID NO: 14 - DNA, 20 bp, Artificial Sequence
  Synthetic Polynucleotide
atggccttccgtgttcctac

SEQ ID NO: 15 - DNA, 19 bp, Artificial Sequence
  Synthetic Polynucleotide
tcaaagcacacgccctctt

SEQ ID NO: 16 - DNA, 20 bp, Artificial Sequence
  Synthetic Polynucleotide
aagcttgctggtgaaaagga

SEQ ID NO: 17 - DNA, 20 bp, Mus musculus
gcaaggagagtggatgggta

SEQ ID NO: 18 - DNA, 18 bp, Homo sapiens
ctacaggccgtgctgctg

SEQ ID NO: 19 - DNA, 21 bp, Artificial Sequence
  Synthetic Polynucleotide
catggtagctgggatgttagg

SEQ ID NO: 20 - DNA, 20 bp, Mus musculus
gtagccacaggtcccttgtc

SEQ ID NO: 21 - DNA, 20 bp, Homo sapiens
aattctgcctctggggtttt

SEQ ID NO: 22 - DNA, 19 bp, Artificial Sequence
  Synthetic Polynucleotide
ctcaccctgggcgttctct

SEQ ID NO: 23 - DNA, 20 bp, Mus musculus
ggtccagtggataagcgaaa

SEQ ID NO: 24 - DNA, 20 bp, Homo sapiens
gactcttccgtgcgttcttc

SEQ ID NO: 25 - DNA, 21 bp, Artificial Sequence
  Synthetic Polynucleotide
atgtcgctttccaacaagctg

SEQ ID NO: 26 - DNA, 20 bp, Mus musculus
taatgtcagcggaacaggac

SEQ ID NO: 27 - DNA, 20 bp, Homo sapiens
atcctggctttggaggctat

SEQ ID NO: 28 - DNA, 20 bp, Mus musculus
atgcctccagctacagccta

SEQ ID NO: 29 - DNA, 20 bp, Homo sapiens
agggagagctggaaaaggag

SEQ ID NO: 30 - DNA, 22 bp, Mus musculus
gtggaagaggaggagagtgaga

SEQ ID NO: 31 - DNA, 20 bp, Homo sapiens
agggactcccgagagcttag

SEQ ID NO: 32 - DNA, 22 bp, Mus musculus
aagtcatacagcagcccaatca

SEQ ID NO: 33 - DNA, 20 bp, Homo sapiens
tgatcagtgcttctgcaacc

SEQ ID NO: 34 - DNA, 20 bp, Artificial Sequence
  Synthetic Polynucleotide
aaaacagctcctccgattcc

SEQ ID NO: 35 - DNA, 21 bp, Artificial Sequence
  Synthetic Polynucleotide
caatctcgcaagatccggtga

SEQ ID NO: 36 - DNA, 20 bp, Artificial Sequence
  Synthetic Polynucleotide
ccctgctagtttcccaatga

SEQ ID NO: 37 - DNA, 20 bp, Artificial Sequence
  Synthetic Polynucleotide
gatgccaacgacacgtctga

SEQ ID NO: 38 - DNA, 24 bp, Homo sapiens
acgctgcatgtgtccttagtagtc

SEQ ID NO: 39 - DNA, 20 bp, Mus musculus
atgacctttcgctcatggac

SEQ ID NO: 40 - DNA, 20 bp, Homo sapiens
ctgaggtgggtggatcactt

SEQ ID NO: 41 - DNA, 19 bp, Mus musculus
gctgatgtcaactgtttcc

SEQ ID NO: 42 - DNA, 20 bp, Homo sapiens
tcgggcaaggacaaagatac

SEQ ID NO: 43 - DNA, 21 bp, Artificial Sequence
  Synthetic Polynucleotide
gccgatccacacggagtactt

SEQ ID NO: 44 - DNA, 20 bp, Mus musculus
ttcccctgctcataaacctg

SEQ ID NO: 45 - DNA, 20 bp, Homo sapiens
cgtttccctgaaccatgact

SEQ ID NO: 46 - DNA, 18 bp, Mus musculus
cctccaactggagctgta

SEQ ID NO: 47 - DNA, 20 bp, Homo sapiens
actgaccacccaaaatctgc

SEQ ID NO: 48 - DNA, 22 bp, Artificial Sequence
  Synthetic Polynucleotide
gctaaccaccaatcttcctttg

SEQ ID NO: 49 - DNA, 23 bp, Artificial Sequence
  Synthetic Polynucleotide
gctgctgttgctgctgctgcttc

SEQ ID NO: 50 - DNA, 24 bp, Mus musculus
actgaaagggtgtcactgtccgac

SEQ ID NO: 51 - DNA, 20 bp, Homo sapiens
tgaaagctgcatgtcctcac

SEQ ID NO: 52 - DNA, 20 bp, Artificial Sequence
  Synthetic Polynucleotide
tttaatagcaccgggcactc

SEQ ID NO: 53 - DNA, 27 bp, Artificial Sequence
  Synthetic Polynucleotide
actctaaactcatacacctgtctacat

SEQ ID NO: 54 - DNA, 20 bp, Mus musculus
atgatggtttctggccactc

SEQ ID NO: 55 - DNA, 20 bp, Homo sapiens
atgtcaatgcctccttggac

SEQ ID NO: 56 - DNA, 20 bp, Artificial Sequence
  Synthetic Polynucleotide
atagggcctctcttgctcag

SEQ ID NO: 57 - DNA, 19 bp, Artificial Sequence
  Synthetic Polynucleotide
tagcgcacagccagtttcc

SEQ ID NO: 58 - DNA, 20 bp, Artificial Sequence
  Synthetic Polynucleotide
ttgcgctcatcttaggcttt

SEQ ID NO: 59 - DNA, 20 bp, Mus musculus
acttgtgatgctgtgcttgc

SEQ ID NO: 60 - DNA, 20 bp, Homo sapiens
ctgactagctggcctccatc

SEQ ID NO: 61 - DNA, 23 bp, Artificial Sequence
  Synthetic Polynucleotide
gcaatcaattctactttagagcg

SEQ ID NO: 62 - DNA, 25 bp, Mus musculus
ctgagaacaagtacacagagagtga

SEQ ID NO: 63 - DNA, 20 bp, Homo sapiens
gctgtttccttcaggagtcg

SEQ ID NO: 64 - DNA, 18 bp, Artificial Sequence
  Synthetic Polynucleotide
aggcctcgaagcgacaga

SEQ ID NO: 65 - DNA, 20 bp, Mus musculus
tttctgcaccacttgtgagc

SEQ ID NO: 66 - DNA, 20 bp, Homo sapiens
gaggagaaaggtgacccaca

SEQ ID NO: 67 - DNA, 21 bp, Artificial Sequence
  Synthetic Polynucleotide
gctccattgtccaagcagaat

SEQ ID NO: 68 - DNA, 20 bp, Mus musculus
ttatctgggcttccgagttg

SEQ ID NO: 69 - DNA, 20 bp, Homo sapiens
gtggcccaaagttaaaagca

SEQ ID NO: 70 - DNA, 20 bp, Mus musculus
gcccaatgctaactgagagc

SEQ ID NO: 71 - DNA, 20 bp, Homo sapiens
agccctccctggtttagtgt

SEQ ID NO: 72 - DNA, 22 bp, Mus musculus
aaattcctcagagtgaggcttg

SEQ ID NO: 73 - DNA, 20 bp, Homo sapiens
ttgttcttgttgctgcttgg

SEQ ID NO: 74 - DNA, 21 bp, Mus musculus
ccagaaggcttcggacaagtc

SEQ ID NO: 75 - DNA, 20 bp, Homo sapiens
tcacaggtggagttttccag

SEQ ID NO: 76 - DNA, 20 bp, Artificial Sequence
  Synthetic Polynucleotide
taaagagccctccatcttgc

SEQ ID NO: 77 - DNA, 22 bp, Artificial Sequence
  Synthetic Polynucleotide
tcaagatgcgtggatatctcgg

SEQ ID NO: 78 - DNA, 20 bp, Artificial Sequence
  Synthetic Polynucleotide
ggaattgagaaagggcacaa

SEQ ID NO: 79 - DNA, 23 bp, Artificial Sequence
  Synthetic Polynucleotide
aaggactccaaagtaacaattca

SEQ ID NO: 80 - DNA, 25 bp, Homo sapiens
atttggagcctcttatagctgtttg

SEQ ID NO: 81 - DNA, 20 bp, Mus musculus
ggcaagctttgctttagtgc

SEQ ID NO: 82 - DNA, 20 bp, Homo sapiens
ctctgcttcctgggttcaag

SEQ ID NO: 83 - DNA, 18 bp, Mus musculus
cgcagaatcttccaccct

SEQ ID NO: 84 - DNA, 20 bp, Homo sapiens
cgatggctatgaagggaaaa

SEQ ID NO: 85 - DNA, 20 bp, Artificial Sequence
  Synthetic Polynucleotide
ccgatctgtgcaggagaccg

SEQ ID NO: 86 - DNA, 20 bp, Artificial Sequence
  Synthetic Polynucleotide
gacccgggagacggtcagca

SEQ ID NO: 87 - DNA, 19 bp, Artificial Sequence
  Synthetic Polynucleotide
tgagcatcccaccccccta

SEQ ID NO: 88 - DNA, 22 bp, Artificial Sequence
  Synthetic Polynucleotide
attgggaacttggggtggaggc

SEQ ID NO: 89 - DNA, 18 bp, Artificial Sequence
  Synthetic Polynucleotide
atgcccactccgtcagcg

SEQ ID NO: 90 - DNA, 20 bp, Artificial Sequence
  Synthetic Polynucleotide
cttcaagcagagcacaaagc

SEQ ID NO: 91 - DNA, 24 bp, Artificial Sequence
  Synthetic Polynucleotide
tggggtcctcggagctctcgggct

SEQ ID NO: 92 - DNA, 23 bp, Artificial Sequence
  Synthetic Polynucleotide
agctctcgggctcaggtggaggt

SEQ ID NO: 93 - DNA, 22 bp, Artificial Sequence
  Synthetic Polynucleotide
ccaaacatcagcgtcagtatag

SEQ ID NO: 94 - DNA, 24 bp, Artificial Sequence
  Synthetic Polynucleotide
ggcacacggtatgagaaaagattg

SEQ ID NO: 95 - DNA, 20 bp, Artificial Sequence
  Synthetic Polynucleotide
gctcatccttgtgaactttg

SEQ ID NO: 96 - DNA, 21 bp, Artificial Sequence
  Synthetic Polynucleotide
gtggcacacgaaaggtttctc

SEQ ID NO: 97 - DNA, 22 bp, Artificial Sequence
  Synthetic Polynucleotide
agagcattacaattcaaggctc

SEQ ID NO: 98 - DNA, 20 bp, Artificial Sequence
  Synthetic Polynucleotide
gatgccaacgacacgtctga

SEQ ID NO: 99 - DNA, 20 bp, Artificial Sequence
  Synthetic Polynucleotide
tgtgagggagatgctcagtg

SEQ ID NO: 100 - DNA, 24 bp, Artificial Sequence
  Synthetic Polynucleotide
taaaggtccaataagatgtcagaa

SEQ ID NO: 101 - DNA, 21 bp, Artificial Sequence
  Synthetic Polynucleotide
gtgctcctgcctcaagaagaa

SEQ ID NO: 102 - DNA, 20 bp, Artificial Sequence
  Synthetic Polynucleotide
ggagagaaaccacggaagaa

SEQ ID NO: 103 - DNA, 25 bp, Artificial Sequence
  Synthetic Polynucleotide
gcactcttcactcctctaaatccag

SEQ ID NO: 104 - DNA, 23 bp, Mus musculus
cttgggcctggatcttggggatc

SEQ ID NO: 105 - DNA, 20 bp, Mus musculus
gggaacttcctgactagggg

SEQ ID NO: 106 - DNA, 20 bp, Mus musculus
agcgcacgaggcggaacaaa

SEQ ID NO: 107 - DNA, 20 bp, Mus musculus
aaaagccagaggtgcaagaa

SEQ ID NO: 108 - DNA, 30 bp, Mus musculus
ttgtctagagagcatggagggccatgtcaa

SEQ ID NO: 109 - DNA, 20 bp, Mus musculus
gggccagttgtgtgacttgg

SEQ ID NO: 110 - DNA, 20 bp, Mus musculus
gggccagttgtgtgacttgg

SEQ ID NO: 111 - DNA, 20 bp, Mus musculus
agagagccgctgtgaggcgt

SEQ ID NO: 112 - DNA, 20 bp, Mus musculus
tatgatcggaattcctcgac

SEQ ID NO: 113 - DNA, 30 bp, Mus musculus
ccactcctctgtgacactttagccctccga

SEQ ID NO: 114 - DNA, 18 bp, Artificial Sequence
  Synthetic Polynucleotide
tccgcctcctcctctgct

SEQ ID NO: 115 - DNA, 20 bp, Artificial Sequence
  Synthetic Polynucleotide
gggaatttattgatttgcat

SEQ ID NO: 116 - DNA, 22 bp, Artificial Sequence
  Synthetic Polynucleotide
ccggccaaaattgatgctttcc

SEQ ID NO: 117 - DNA, 24 bp, Artificial Sequence
  Synthetic Polynucleotide
cagtcccaaaagcatcattgacat

SEQ ID NO: 118 - DNA, 16 bp, Artificial Sequence
  Synthetic Polynucleotide
cactgtccaaactagg

SEQ ID NO: 119 - DNA, 16 bp, Artificial Sequence
  Synthetic Polynucleotide
cactgtccacactagg